European Patent Specification EP 3 858 979 B1, published September 2, 2026. Title: METHODS AND COMPOSITIONS FOR PREPARING CARDIOMYOCYTES FROM STEM CELLS AND USES THEREOF. Applicant: INSTITUTE OF BIOPHYSICS, CHINESE ACADEMY OF SCIENCES MA, Yue. Application EP 10853137.7. The sequence listing filed with the application follows.

SEQUENCE LISTING (8 sequences)

SEQ ID NO: 1 - DNA, 22 bp, Artificial Sequence
  forward primer
acctcaacagctccctgactct

SEQ ID NO: 2 - DNA, 23 bp, Artificial Sequence
  reverse primer
ataatcgccgccacaaactctcc

SEQ ID NO: 3 - DNA, 24 bp, Artificial Sequence
  forward primer
ttcaccaaagatctgctcctcgct

SEQ ID NO: 4 - DNA, 26 bp, Artificial Sequence
  reverse primer
ttattactggtgtggagtgggtgtgg

SEQ ID NO: 5 - DNA, 20 bp, Artificial Sequence
  forward primer
ttccgttctgaagcgtggtc

SEQ ID NO: 6 - DNA, 22 bp, Artificial Sequence
  reverse primer
tgaagcaggcaattattggtgt

SEQ ID NO: 7 - DNA, 24 bp, Artificial Sequence
  forward primer
gaaatcccatcaccatcttccagg

SEQ ID NO: 8 - DNA, 20 bp, Artificial Sequence
  reverse primer
gagccccagccttctccatg